European Patent Application EP 4 226 942 A1, published August 16, 2023. Title: USE OF ANTI-PD-1 ANTIBODY IN COMBINATION THERAPY. Applicant: BIO-THERA SOLUTIONS, LTD. Application EP21877032.9. The sequence listing filed with the application follows.

SEQUENCE LISTING (18 sequences)

SEQ ID NO: 1 - protein, 6 aa, Artificial Sequence
  HCDR1 of antibody A
NYYMYW

SEQ ID NO: 2 - protein, 15 aa, Artificial Sequence
  HCDR2 of antibody A
GINPSNGGTNFNEKF

SEQ ID NO: 3 - protein, 12 aa, Artificial Sequence
  HCDR3 of antibody A
ARDYRLDMGFEF

SEQ ID NO: 4 - protein, 14 aa, Artificial Sequence
  LCDR1 of antibody A
ASKGVSTSGYSYLH

SEQ ID NO: 5 - protein, 6 aa, Artificial Sequence
  LCDR2 of antibody A
LASYLE

SEQ ID NO: 6 - protein, 11 aa, Artificial Sequence
  LCDR3 of antibody A
YCQHAYDLPLT

SEQ ID NO: 7 - protein, 120 aa, Artificial Sequence
  VH of antibody A
QVQLVQSGVEVKKPGASVKVSCKASGYTFTNYYMYWVRQAPGQGLEWMGGINPSNGGTNFNEKFKNRVTLTTDSSTTTAYMELKSLQFDDTAVYYCAARDYRLDMGFEFWGQGTTVTVSS

SEQ ID NO: 8 - protein, 111 aa, Artificial Sequence
  VL of antibody A
EIVLTQSPATLSLSPGERATLSCRASKGVSTSGYSYLHWYQQKPGQAPRLLIYLASYLESGVPARFSGSGSGTDFTLTISSLEPEDFAVYYCQHAYDLPLTFGGGTKVEIK

SEQ ID NO: 9 - protein, 447 aa, Artificial Sequence
  Heavy chain of antibody A
QVQLVQSGVEVKKPGASVKVSCKASGYTFTNYYMYWVRQAPGQGLEWMGGINPSNGGTNFNEKFKNRVTLTTDSSTTTAYMELKSLQFDDTAVYYCAARDYRLDMGFEFWGQGTTVTVSSASTKGPSVFPLAPCSRSTSESTAALGCLVKDYFPEPVTVSWNSGALTSGVHTFPAVLQSSGLYSLSSVVTVPSSSLGTKTYTCNVDHKPSNTKVDKRVESKYGPPCPPCPAPEFLGGPSVFLFPPKPKDTLMISRTPEVTCVVVDVSQEDPEVQFNWYVDGVEVHNAKTKPREEQFNSTYRVVSVLTVLHQDWLNGKEYKCKVSNKGLPSSIEKTISKAKGQPREPQVYTLPPSQEEMTKNQVSLTCLVKGFYPSDIAVEWESNGQPENNYKTTPPVLDSDGSFFLYSRLTVDKSRWQEGNVFSCSVMHEALHNHYTQKSLSLSLGK

SEQ ID NO: 10 - protein, 218 aa, Artificial Sequence
  Light chain of antibody A
EIVLTQSPATLSLSPGERATLSCRASKGVSTSGYSYLHWYQQKPGQAPRLLIYLASYLESGVPARFSGSGSGTDFTLTISSLEPEDFAVYYCQHAYDLPLTFGGGTKVEIKRTVAAPSVFIFPPSDEQLKSGTASVVCLLNNFYPREAKVQWKVDNALQSGNSQESVTEQDSKDSTYSLSSTLTLSKADYEKHKVYACEVTHQGLSSPVTKSFNRGEC

SEQ ID NO: 11 - protein, 450 aa, Artificial Sequence
  Heavy chain of antibody B
EVQLVESGGGLVQPGGSLRLSCAASGFNIKDTYIHWVRQAPGKGLEWVARIYPTNGYTRYADSVKGRFTISADTSKNTAYLQMNSLRAEDTAVYYCSRWGGDGFYAMDYWGQGTLVTVSSASTKGPSVFPLAPSSKSTSGGTAALGCLVKDYFPEPVTVSWNSGALTSGVHTFPAVLQSSGLYSLSSVVTVPSSSLGTQTYICNVNHKPSNTKVDKKVEPKSCDKTHTCPPCPAPELLGGPSVFLFPPKPKDTLMISRTPEVTCVVVDVSHEDPEVKFNWYVDGVEVHNAKTKPREEQYNSTYRVVSVLTVLHQDWLNGKEYKCKVSNKALPAPIEKTISKAKGQPREPQVYTLPPSREEMTKNQVSLTCLVKGFYPSDIAVEWESNGQPENNYKTTPPVLDSDGSFFLYSKLTVDKSRWQQGNVFSCSVMHEALHNHYTQKSLSLSPGK

SEQ ID NO: 12 - protein, 214 aa, Artificial Sequence
  Light chain of antibody B
DIQMTQSPSSLSASVGDRVTITCRASQDVNTAVAWYQQKPGKAPKLLIYSASFLYSGVPSRFSGSRSGTDFTLTISSLQPEDFATYYCQQHYTTPPTFGQGTKVEIKRTVAAPSVFIFPPSDEQLKSGTASVVCLLNNFYPREAKVQWKVDNALQSGNSQESVTEQDSKDSTYSLSSTLTLSKADYEKHKVYACEVTHQGLSSPVTKSFNRGEC

SEQ ID NO: 13 - DNA, 1341 bp, Artificial Sequence
  Heavy chain of antibody A
caggtgcagctggtgcagtccggcgtggaggtgaagaagcctggcgccagcgtgaaggtgtcctgtaaggccagcggctacaccttcaccaattactatatgtattgggtgcggcaggcccccggccagggactggagtggatgggaggcatcaatcccagcaacggcggcaccaacttcaatgagaagtttaagaaccgggtgaccctgaccaccgatagcagcaccaccaccgcttacatggagctgaagagcctgcagtttgacgataccgctgtgtactattgcgctgcccgggattacaggctggacatgggcttcgagttctggggccagggcaccaccgtgaccgtgtccagcgctagcaccaagggcccttccgtgttccccctggccccctgtagccggtccacctctgagagcaccgctgctctgggctgtctggtgaaggattactttcccgaaccggtgaccgtgtcatggaactccggggctctgacatccggtgtccacacttttcctgcagtgctgcagtcatccggcctgtacagcctgagctctgtggtcacagtcccaagttcatccctgggaaccaagacatatacttgcaacgtggatcataaacccagcaatactaaggtcgacaaacgagtggagtctaagtacggaccaccttgcccaccatgtccagcacctgagttcctgggaggaccaagcgtgttcctgtttcctccaaagcctaaagataccctgatgatcagtcggactcccgaggtcacctgcgtggtcgtggacgtgtcccaggaggaccctgaagtccagttcaactggtacgtggacggcgtcgaagtgcacaatgctaagacaaaacctcgagaggaacagtttaactccacataccgtgtcgtgagcgtcctgactgtgctgcatcaggattggctgaacggcaaggagtataagtgcaaagtgagcaataagggactgccaagctctatcgagaaaactatttctaaggctaaaggacagcctagggaaccacaggtgtacaccctgccccctagtcaggaggaaatgactaagaaccaggtctcactgacctgtctggtgaaagggttctatccttcagatattgcagtggagtgggaatccaatggtcagccagagaacaattacaagacaactccacccgtgctggacagcgatgggtctttctttctgtattctagactgaccgtggacaaaagtcgctggcaggagggtaatgtcttttcttgtagtgtgatgcacgaagccctgcacaaccactacactcagaaaagcctgtcactgtccctgggtaaa

SEQ ID NO: 14 - DNA, 654 bp, Artificial Sequence
  Light chain of antibody A
gagatcgtgctgacccagtcccccgctaccctgagcctgtcccccggagagcgggctaccctgtcttgtcgggcctccaagggcgtgagcaccagcggatactcctatctgcactggtaccagcagaagcccggccaggctcccaggctgctgatctacctggcttcctacctggagagcggcgtgcccgctaggtttagcggcagcggcagcggaaccgatttcaccctgaccatcagctccctggagcccgaggattttgccgtgtactactgccagcacgcttacgacctgcccctgacctttggcggcggcaccaaggtggagatcaagcgtacggtggctgcaccatctgtcttcatcttcccgccatctgatgagcagttgaaatctggaactgcctctgttgtgtgcctgctgaataacttctatcccagagaggccaaagtacagtggaaggtggataacgccctccaatcgggtaactcccaggagagtgtcacagagcaggacagcaaggacagcacctacagcctcagcagcaccctgacgctgagcaaagcagactacgagaaacacaaagtctacgcctgcgaagtcacccatcagggcctgagctcgcccgtcacaaagagcttcaacaggggagagtgt

SEQ ID NO: 15 - protein, 448 aa, Artificial Sequence
  Heavy chain of antibody C
QVQLVESGGGVVQPGRSLRLSCAASGFTFSSYTMHWVRQAPGKGLEWVTFISYDGNNKYYADSVKGRFTISRDNSKNTLYLQMNSLRAEDTAIYYCARTGWLGPFDYWGQGTLVTVSSASTKGPSVFPLAPSSKSTSGGTAALGCLVKDYFPEPVTVSWNSGALTSGVHTFPAVLQSSGLYSLSSVVTVPSSSLGTQTYICNVNHKPSNTKVDKRVEPKSCDKTHTCPPCPAPELLGGPSVFLFPPKPKDTLMISRTPEVTCVVVDVSHEDPEVKFNWYVDGVEVHNAKTKPREEQYNSTYRVVSVLTVLHQDWLNGKEYKCKVSNKALPAPIEKTISKAKGQPREPQVYTLPPSRDELTKNQVSLTCLVKGFYPSDIAVEWESNGQPENNYKTTPPVLDSDGSFFLYSKLTVDKSRWQQGNVFSCSVMHEALHNHYTQKSLSLSPGK

SEQ ID NO: 16 - protein, 215 aa, Artificial Sequence
  Light chain of antibody C
EIVLTQSPGTLSLSPGERATLSCRASQSVGSSYLAWYQQKPGQAPRLLIYGAFSRATGIPDRFSGSGSGTDFTLTISRLEPEDFAVYYCQQYGSSPWTFGQGTKVEIKRTVAAPSVFIFPPSDEQLKSGTASVVCLLNNFYPREAKVQWKVDNALQSGNSQESVTEQDSKDSTYSLSSTLTLSKADYEKHKVYACEVTHQGLSSPVTKSFNRGEC

SEQ ID NO: 17 - DNA, 1344 bp, Artificial Sequence
  Heavy chain of antibody C
caggtccagctggtcgaatctggcggcggcgtcgtccagcctggaagatctctgagactgtcttgcgctgcttctggctttaccttctcttcttacacaatgcattgggtcagacaggctcctggtaaaggtctggagtgggtcacattcatctcttacgacggcaacaacaagtactacgccgattctgtcaagggcagattcaccatctccagagacaactccaagaacaccctgtacctgcagatgaactctctgagagctgaggataccgctatctactattgcgctagaacaggctggctgggaccttttgattactggggacagggaacactggtcacagtctcttctgcttctaccaaaggaccttctgtctttcctctggctccttcttctaagtctacctctggcggaacagctgctctgggttgtctggtcaaggattacttccctgaaccggtgacagtgtcttggaattctggagctctgacctcaggagtccatacatttcctgctgtcctgcagtcttctggcctgtattctctgtcctctgtggtgacagtcccttcttcttctctgggaacacagacctacatctgcaacgtcaaccacaagccttccaacaccaaggtcgacaagagagtggagcctaagtcttgcgacaagacacatacatgtccaccgtgcccagcacctgaactcctggggggaccgtcagtcttcctcttccccccaaaacccaaggacaccctcatgatctcccggacccctgaggtcacatgcgtggtggtggacgtgagccacgaagaccctgaggtcaagttcaactggtacgtggacggcgtggaggtgcataatgccaagacaaagccgcgggaggagcagtacaacagcacgtaccgtgtggtcagcgtcctcaccgtcctgcaccaggactggctgaatggcaaggagtacaagtgcaaggtctccaacaaagccctcccagcccccatcgagaaaaccatctccaaagccaaagggcagccccgagaaccacaggtgtacaccctgcccccatcccgggatgagctgaccaagaaccaggtcagcctgacctgcctggtcaaaggcttctatcccagcgacatcgccgtggagtgggagagcaatgggcagccggagaacaactacaagaccacgcctcccgtgctggactccgacggctccttcttcctctacagcaagctcaccgtggacaagagcaggtggcagcaggggaacgtcttctcatgctccgtgatgcatgaggctctgcacaaccactacacgcagaagagcctctccctgtctccgggtaaa

SEQ ID NO: 18 - DNA, 645 bp, Artificial Sequence
  Light chain of antibody C
gaaattgtcctgacacagtctcctggaacactgtctctgtctcctggagagagagctacactgtcttgtagggcttctcagtctgtgggatcttcttacctggcttggtatcagcagaaacctggacaggctcctagactgctgatctacggcgctttttctagagctaccggaatccctgacagattctctggatctggctctggaaccgatttcaccctgaccatctctagactggaacctgaggactttgctgtctactactgtcagcagtacggctcttctccttggacatttggacagggaaccaaggtcgagatcaagcgtacggtggctgcaccatctgtcttcatcttcccgccatctgatgagcagttgaaatctggaactgcctctgttgtgtgcctgctgaataacttctatcccagagaggccaaagtacagtggaaggtggataacgccctccaatcgggtaactcccaggagagtgtcacagagcaggacagcaaggacagcacctacagcctcagcagcaccctgacgctgagcaaagcagactacgagaaacacaaagtctacgcctgcgaagtcacccatcagggcctgagctcgcccgtcacaaagagcttcaacaggggagagtgt